European Patent Application EP 4 249 481 A1, published September 27, 2023. Title: Dihydroisoquinolinone and Isoindolinone Derivatives and Uses Thereof. Applicant: HEFEI INSTITUTES OF PHYSICAL SCIENCE, CHINESE ACADEMY OF SCIENCES. The sequence listing filed with the application follows.

SEQUENCE LISTING (2 sequences)

SEQ ID NO: 1 - DNA, 6856 bp, Artificial Sequence
gacggatcgggagatctcccgatcccctatggtgcactctcagtacaatctgctctgatgccgcatagttaagccagtatctgctccctgcttgtgtgttggaggtcgctgagtagtgcgcgagcaaaatttaagctacaacaaggcaaggcttgaccgacaattgcatgaagaatctgcttagggttaggcgttttgcgctgcttcgcgatgtacgggccagatatacgcgttgacattgattattgactagttattaatagtaatcaattacggggtcattagttcatagcccatatatggagttccgcgttacataacttacggtaaatggcccgcctggctgaccgcccaacgacccccgcccattgacgtcaataatgacgtatgttcccatagtaacgccaatagggactttccattgacgtcaatgggtggagtatttacggtaaactgcccacttggcagtacatcaagtgtatcatatgccaagtacgccccctattgacgtcaatgacggtaaatggcccgcctggcattatgcccagtacatgaccttatgggactttcctacttggcagtacatctacgtattagtcatcgctattaccatggtgatgcggttttggcagtacatcaatgggcgtggatagcggtttgactcacggggatttccaagtctccaccccattgacgtcaatgggagtttgttttggcaccaaaatcaacgggactttccaaaatgtcgtaacaactccgccccattgacgcaaatgggcggtaggcgtgtacggtgggaggtctatataagcagagctctctggctaactagagaacccactgcttactggcttatcgaaattaatacgactcactatagggagacccaagctggctagcgccaccatggtggactacagcgtgtgggaccacattgaggtgtctgatgatgaagacgagacgcaccccaacatcgacacggccagtctcttccgctggcggcatcaggcccgggtggaacgcatggagcagttccagaaggagaaggaggaactggacaggggctgccgcgagtgcaagcgcaaggtggccgagtgccagaggaaactgaaggagctggaggtggccgagggcggcaaggcagagctggagcgcctgcaggccgaggcacagcagctgcgcaaggaggagcggagctgggagcagaagctggaggagatgcgcaagaaggagaagagcatgccctggaacgtggacacgctcagcaaagacggcttcagcaagagcatggtaaataccaagcccgagaagacggaggaggactcagaggaggtgagggagcagaaacacaagaccttcgtggaaaaatacgagaaacagatcaagcactttggcatgcttcgccgctgggatgacagccaaaagtacctgtcagacaacgtccacctggtgtgcgaggagacagccaattacctggtcatttggtgcattgacctagaggtggaggagaaatgtgcactcatggagcaggtggcccaccagacaatcgtcatgcaatttatcctggagctggccaagagcctaaaggtggacccccgggcctgcttccggcagttcttcactaagattaagacagccgatcgccagtacatggagggcttcaacgacgagctggaagccttcaaggagcgtgtgcggggccgtgccaagctgcgcatcgagaaggccatgaaggagtacgaggaggaggagcgcaagaagcggctcggccccggcggcctggaccccgtcgaggtctacgagtccctccctgaggaactccagaagtgcttcgatgtgaaggacgtgcagatgctgcaggacgccatcagcaagatggaccccaccgacgcaaagtaccacatgcagcgctgcattgactctggcctctgggtccccaactctaaggccagcgaggccaaggagggagaggaggcaggtcctggggacccattactggaagctgttcccaagacgggcgatgagaaggatgtcagtgtgaagcttggtaccgagctcggatccggtggcggagggagcggtggcggagggagcggcggccgcaagcccgacgtcgtccagattgtccgcaactacaacgcctaccttcgggccagcgacgatctgcctaagatgttcatcgagtccgaccctgggttcttttccaacgctattgtcgagggagctaagaagttccctaacaccgagttcgtgaaggtgaagggcctccacttcagccaggaggacgctccagatgaaatgggtaagtacatcaagagcttcgtggagcgcgtgctgaagaacgagcagagtctagaggctgactacaaagaccatgacggtgattataaagatcatgacatcgactacaaggatgacgatgacaagtgagtttaaacccgctgatcagcctcgactgtgccttctagttgccagccatctgttgtttgcccctcccccgtgccttccttgaccctggaaggtgccactcccactgtcctttcctaataaaatgaggaaattgcatcgcattgtctgagtaggtgtcattctattctggggggtggggtggggcaggacagcaagggggaggattgggaagacaatagcaggcatgctggggatgcggtgggctctatggcttctgaggcggaaagaaccagctggggctctagggggtatccccacgcgccctgtagcggcgcattaagcgcggcgggtgtggtggttacgcgcagcgtgaccgctacacttgccagcgccctagcgcccgctcctttcgctttcttcccttcctttctcgccacgttcgccggctttccccgtcaagctctaaatcgggggctccctttagggttccgatttagtgctttacggcacctcgaccccaaaaaacttgattagggtgatggttcacgtagtgggccatcgccctgatagacggtttttcgccctttgacgttggagtccacgttctttaatagtggactcttgttccaaactggaacaacactcaaccctatctcggtctattcttttgatttataagggattttgccgatttcggcctattggttaaaaaatgagctgatttaacaaaaatttaacgcgaattaattctgtggaatgtgtgtcagttagggtgtggaaagtccccaggctccccagcaggcagaagtatgcaaagcatgcatctcaattagtcagcaaccaggtgtggaaagtccccaggctccccagcaggcagaagtatgcaaagcatgcatctcaattagtcagcaaccatagtcccgcccctaactccgcccatcccgcccctaactccgcccagttccgcccattctccgccccatggctgactaattttttttatttatgcagaggccgaggccgcctctgcctctgagctattccagaagtagtgaggaggcttttttggaggcctaggcttttgcaaaaagctcccgggagcttgtatatccattttcggatctgatcaagagacaggatgaggatcgtttcgcatgattgaacaagatggattgcacgcaggttctccggccgcttgggtggagaggctattcggctatgactgggcacaacagacaatcggctgctctgatgccgccgtgttccggctgtcagcgcaggggcgcccggttctttttgtcaagaccgacctgtccggtgccctgaatgaactgcaggacgaggcagcgcggctatcgtggctggccacgacgggcgttccttgcgcagctgtgctcgacgttgtcactgaagcgggaagggactggctgctattgggcgaagtgccggggcaggatctcctgtcatctcaccttgctcctgccgagaaagtatccatcatggctgatgcaatgcggcggctgcatacgcttgatccggctacctgcccattcgaccaccaagcgaaacatcgcatcgagcgagcacgtactcggatggaagccggtcttgtcgatcaggatgatctggacgaagagcatcaggggctcgcgccagccgaactgttcgccaggctcaaggcgcgcatgcccgacggcgaggatctcgtcgtgacccatggcgatgcctgcttgccgaatatcatggtggaaaatggccgcttttctggattcatcgactgtggccggctgggtgtggcggaccgctatcaggacatagcgttggctacccgtgatattgctgaagagcttggcggcgaatgggctgaccgcttcctcgtgctttacggtatcgccgctcccgattcgcagcgcatcgccttctatcgccttcttgacgagttcttctgagcgggactctggggttcgaaatgaccgaccaagcgacgcccaacctgccatcacgagatttcgattccaccgccgccttctatgaaaggttgggcttcggaatcgttttccgggacgccggctggatgatcctccagcgcggggatctcatgctggagttcttcgcccaccccaacttgtttattgcagcttataatggttacaaataaagcaatagcatcacaaatttcacaaataaagcatttttttcactgcattctagttgtggtttgtccaaactcatcaatgtatcttatcatgtctgtataccgtcgacctctagctagagcttggcgtaatcatggtcatagctgtttcctgtgtgaaattgttatccgctcacaattccacacaacatacgagccggaagcataaagtgtaaagcctggggtgcctaatgagtgagctaactcacattaattgcgttgcgctcactgcccgctttccagtcgggaaacctgtcgtgccagctgcattaatgaatcggccaacgcgcggggagaggcggtttgcgtattgggcgctcttccgcttcctcgctcactgactcgctgcgctcggtcgttcggctgcggcgagcggtatcagctcactcaaaggcggtaatacggttatccacagaatcaggggataacgcaggaaagaacatgtgagcaaaaggccagcaaaaggccaggaaccgtaaaaaggccgcgttgctggcgtttttccataggctccgcccccctgacgagcatcacaaaaatcgacgctcaagtcagaggtggcgaaacccgacaggactataaagataccaggcgtttccccctggaagctccctcgtgcgctctcctgttccgaccctgccgcttaccggatacctgtccgcctttctcccttcgggaagcgtggcgctttctcatagctcacgctgtaggtatctcagttcggtgtaggtcgttcgctccaagctgggctgtgtgcacgaaccccccgttcagcccgaccgctgcgccttatccggtaactatcgtcttgagtccaacccggtaagacacgacttatcgccactggcagcagccactggtaacaggattagcagagcgaggtatgtaggcggtgctacagagttcttgaagtggtggcctaactacggctacactagaagaacagtatttggtatctgcgctctgctgaagccagttaccttcggaaaaagagttggtagctcttgatccggcaaacaaaccaccgctggtagcggtttttttgtttgcaagcagcagattacgcgcagaaaaaaaggatctcaagaagatcctttgatcttttctacggggtctgacgctcagtggaacgaaaactcacgttaagggattttggtcatgagattatcaaaaaggatcttcacctagatccttttaaattaaaaatgaagttttaaatcaatctaaagtatatatgagtaaacttggtctgacagttaccaatgcttaatcagtgaggcacctatctcagcgatctgtctatttcgttcatccatagttgcctgactccccgtcgtgtagataactacgatacgggagggcttaccatctggccccagtgctgcaatgataccgcgagacccacgctcaccggctccagatttatcagcaataaaccagccagccggaagggccgagcgcagaagtggtcctgcaactttatccgcctccatccagtctattaattgttgccgggaagctagagtaagtagttcgccagttaatagtttgcgcaacgttgttgccattgctacaggcatcgtggtgtcacgctcgtcgtttggtatggcttcattcagctccggttcccaacgatcaaggcgagttacatgatcccccatgttgtgcaaaaaagcggttagctccttcggtcctccgatcgttgtcagaagtaagttggccgcagtgttatcactcatggttatggcagcactgcataattctcttactgtcatgccatccgtaagatgcttttctgtgactggtgagtactcaaccaagtcattctgagaatagtgtatgcggcgaccgagttgctcttgcccggcgtcaatacgggataataccgcgccacatagcagaactttaaaagtgctcatcattggaaaacgttcttcggggcgaaaactctcaaggatcttaccgctgttgagatccagttcgatgtaacccactcgtgcacccaactgatcttcagcatcttttactttcaccagcgtttctgggtgagcaaaaacaggaaggcaaaatgccgcaaaaaagggaataagggcgacacggaaatgttgaatactcatactcttcctttttcaatattattgaagcatttatcagggttattgtctcatgagcggatacatatttgaatgtatttagaaaaataaacaaataggggttccgcgcacatttccccgaaaagtgccacctgacgtc

SEQ ID NO: 2 - DNA, 7338 bp, Artificial Sequence
gacggatcgggagatctcccgatcccctatggtgcactctcagtacaatctgctctgatgccgcatagttaagccagtatctgctccctgcttgtgtgttggaggtcgctgagtagtgcgcgagcaaaatttaagctacaacaaggcaaggcttgaccgacaattgcatgaagaatctgcttagggttaggcgttttgcgctgcttcgcgatgtacgggccagatatacgcgttgacattgattattgactagttattaatagtaatcaattacggggtcattagttcatagcccatatatggagttccgcgttacataacttacggtaaatggcccgcctggctgaccgcccaacgacccccgcccattgacgtcaataatgacgtatgttcccatagtaacgccaatagggactttccattgacgtcaatgggtggagtatttacggtaaactgcccacttggcagtacatcaagtgtatcatatgccaagtacgccccctattgacgtcaatgacggtaaatggcccgcctggcattatgcccagtacatgaccttatgggactttcctacttggcagtacatctacgtattagtcatcgctattaccatggtgatgcggttttggcagtacatcaatgggcgtggatagcggtttgactcacggggatttccaagtctccaccccattgacgtcaatgggagtttgttttggcaccaaaatcaacgggactttccaaaatgtcgtaacaactccgccccattgacgcaaatgggcggtaggcgtgtacggtgggaggtctatataagcagagctctctggctaactagagaacccactgcttactggcttatcgaaattaatacgactcactatagggagacccaagctggctagcgccaccatggcttccaaggtgtacgaccccgagcaacgcaaacgcatgatcactgggcctcagtggtgggctcgctgcaagcaaatgaacgtgctggactccttcatcaactactatgattccgagaagcacgccgagaacgccgtgatttttctgcatggtaacgctgcctccagctacctgtggaggcacgtcgtgcctcacatcgagcccgtggctagatgcatcatccctgatctgatcggaatgggtaagtccggcaagagcgggaatggctcatatcgcctcctggatcactacaagtacctcaccgcttggttcgagctgctgaaccttccaaagaaaatcatctttgtgggccacgactggggggcttgtctggcctttcactactcctacgagcaccaagacaagatcaaggccatcgtccatgctgagagtgtcgtggacgtgatcgagtcctgggacgagtggcctgacatcgaggaggatatcgccctgatcaagagcgaagagggcgagaaaatggtgcttgagaataacttcttcgtcgagaccatgctcccaagcaagatcatgcggaaactggagcctgaggagttcgctgcctacctggagccattcaaggagaagggcgaggttagacggcctaccctctcctggcctcgcgagatccctctcgttaagggaggcggtggcggagggagcggtggcggagggagcaagcttggtaccgagctcggatccactagatctgttaacgtgtggtggaattctatggcaaagcagtacgactcggtggagtgccctttttgtgatgaagtttccaaatacgagaagctcgccaagatcggccaaggcaccttcggggaggtgttcaaggccaggcaccgcaagaccggccagaaggtggctctgaagaaggtgctgatggaaaacgagaaggaggggttccccattacagccttgcgggagatcaagatccttagcttctaaaacacgagaatgtggtcaacttgattgagatttgtcgaaccaaagcttccccctataaccgctgcaagggtagtatatacctggtgttcgacttctgcgagcatgaccttgctgggctgttgagcaatgttttggtcaagttcacgctgtctgagatcaagagggtgatgcagatgctgcttaacggcctctactacatccacagaaacaagatcctgcatagggacatgaaggctgctaatgtgcttatcactcgtgatggggtcctgaagctggcagactttgggctggcccgggccttcagcctggccaagaacagccagcccaaccgctacaccaaccgtgtggtgacactctggtaccggcccccggagctgttgctcggggagcgggactacggcccccccattgacctgtggggtgctgggtgcatcatggcagagatgtggacccgcagccccatcatgcagggcaacacggagcagcaccaactcgccctcatcagtcagctctgcggctccatcacccctgaggtgtggccaaacgtggacaactatgagctgtacgaaaagctggagctggtcaagggccagaagcggaaggtgaaggacaggctgaaggcctatgtgcgtgacccatacgcactggacctcatcgacaagctgctggtgctggaccctgcccagcgcatcgacagcgatgacgccctcaaccacgacttcttctggtccgaccccatgccctccgacctcaagggcatgctctccacccacctgacgtccatgttcgagtacttggcaccaccgcgccggaagggcagccagatcacccagcagtccaccaaccagagtcgcaatcccgccaccaccaaccagacggagtttgagcgcgtcttctggaattctgcagatatccagcacagtggcggccgctcgagtctagaggctgactacaaagaccatgacggtgattataaagatcatgacatcgactacaaggatgacgatgacaagtgagtttaaacccgctgatcagcctcgactgtgccttctagttgccagccatctgttgtttgcccctcccccgtgccttccttgaccctggaaggtgccactcccactgtcctttcctaataaaatgaggaaattgcatcgcattgtctgagtaggtgtcattctattctggggggtggggtggggcaggacagcaagggggaggattgggaagacaatagcaggcatgctggggatgcggtgggctctatggcttctgaggcggaaagaaccagctggggctctagggggtatccccacgcgccctgtagcggcgcattaagcgcggcgggtgtggtggttacgcgcagcgtgaccgctacacttgccagcgccctagcgcccgctcctttcgctttcttcccttcctttctcgccacgttcgccggctttccccgtcaagctctaaatcgggggctccctttagggttccgatttagtgctttacggcacctcgaccccaaaaaacttgattagggtgatggttcacgtagtgggccatcgccctgatagacggtttttcgccctttgacgttggagtccacgttctttaatagtggactcttgttccaaactggaacaacactcaaccctatctcggtctattcttttgatttataagggattttgccgatttcggcctattggttaaaaaatgagctgatttaacaaaaatttaacgcgaattaattctgtggaatgtgtgtcagttagggtgtggaaagtccccaggctccccagcaggcagaagtatgcaaagcatgcatctcaattagtcagcaaccaggtgtggaaagtccccaggctccccagcaggcagaagtatgcaaagcatgcatctcaattagtcagcaaccatagtcccgcccctaactccgcccatcccgcccctaactccgcccagttccgcccattctccgccccatggctgactaattttttttatttatgcagaggccgaggccgcctctgcctctgagctattccagaagtagtgaggaggcttttttggaggcctaggcttttgcaaaaagctcccgggagcttgtatatccattttcggatctgatcaagagacaggatgaggatcgtttcgcatgattgaacaagatggattgcacgcaggttctccggccgcttgggtggagaggctattcggctatgactgggcacaacagacaatcggctgctctgatgccgccgtgttccggctgtcagcgcaggggcgcccggttctttttgtcaagaccgacctgtccggtgccctgaatgaactgcaggacgaggcagcgcggctatcgtggctggccacgacgggcgttccttgcgcagctgtgctcgacgttgtcactgaagcgggaagggactggctgctattgggcgaagtgccggggcaggatctcctgtcatctcaccttgctcctgccgagaaagtatccatcatggctgatgcaatgcggcggctgcatacgcttgatccggctacctgcccattcgaccaccaagcgaaacatcgcatcgagcgagcacgtactcggatggaagccggtcttgtcgatcaggatgatctggacgaagagcatcaggggctcgcgccagccgaactgttcgccaggctcaaggcgcgcatgcccgacggcgaggatctcgtcgtgacccatggcgatgcctgcttgccgaatatcatggtggaaaatggccgcttttctggattcatcgactgtggccggctgggtgtggcggaccgctatcaggacatagcgttggctacccgtgatattgctgaagagcttggcggcgaatgggctgaccgcttcctcgtgctttacggtatcgccgctcccgattcgcagcgcatcgccttctatcgccttcttgacgagttcttctgagcgggactctggggttcgaaatgaccgaccaagcgacgcccaacctgccatcacgagatttcgattccaccgccgccttctatgaaaggttgggcttcggaatcgttttccgggacgccggctggatgatcctccagcgcggggatctcatgctggagttcttcgcccaccccaacttgtttattgcagcttataatggttacaaataaagcaatagcatcacaaatttcacaaataaagcatttttttcactgcattctagttgtggtttgtccaaactcatcaatgtatcttatcatgtctgtataccgtcgacctctagctagagcttggcgtaatcatggtcatagctgtttcctgtgtgaaattgttatccgctcacaattccacacaacatacgagccggaagcataaagtgtaaagcctggggtgcctaatgagtgagctaactcacattaattgcgttgcgctcactgcccgctttccagtcgggaaacctgtcgtgccagctgcattaatgaatcggccaacgcgcggggagaggcggtttgcgtattgggcgctcttccgcttcctcgctcactgactcgctgcgctcggtcgttcggctgcggcgagcggtatcagctcactcaaaggcggtaatacggttatccacagaatcaggggataacgcaggaaagaacatgtgagcaaaaggccagcaaaaggccaggaaccgtaaaaaggccgcgttgctggcgtttttccataggctccgcccccctgacgagcatcacaaaaatcgacgctcaagtcagaggtggcgaaacccgacaggactataaagataccaggcgtttccccctggaagctccctcgtgcgctctcctgttccgaccctgccgcttaccggatacctgtccgcctttctcccttcgggaagcgtggcgctttctcatagctcacgctgtaggtatctcagttcggtgtaggtcgttcgctccaagctgggctgtgtgcacgaaccccccgttcagcccgaccgctgcgccttatccggtaactatcgtcttgagtccaacccggtaagacacgacttatcgccactggcagcagccactggtaacaggattagcagagcgaggtatgtaggcggtgctacagagttcttgaagtggtggcctaactacggctacactagaagaacagtatttggtatctgcgctctgctgaagccagttaccttcggaaaaagagttggtagctcttgatccggcaaacaaaccaccgctggtagcggtttttttgtttgcaagcagcagattacgcgcagaaaaaaaggatctcaagaagatcctttgatcttttctacggggtctgacgctcagtggaacgaaaactcacgttaagggattttggtcatgagattatcaaaaaggatcttcacctagatccttttaaattaaaaatgaagttttaaatcaatctaaagtatatatgagtaaacttggtctgacagttaccaatgcttaatcagtgaggcacctatctcagcgatctgtctatttcgttcatccatagttgcctgactccccgtcgtgtagataactacgatacgggagggcttaccatctggccccagtgctgcaatgataccgcgagacccacgctcaccggctccagatttatcagcaataaaccagccagccggaagggccgagcgcagaagtggtcctgcaactttatccgcctccatccagtctattaattgttgccgggaagctagagtaagtagttcgccagttaatagtttgcgcaacgttgttgccattgctacaggcatcgtggtgtcacgctcgtcgtttggtatggcttcattcagctccggttcccaacgatcaaggcgagttacatgatcccccatgttgtgcaaaaaagcggttagctccttcggtcctccgatcgttgtcagaagtaagttggccgcagtgttatcactcatggttatggcagcactgcataattctcttactgtcatgccatccgtaagatgcttttctgtgactggtgagtactcaaccaagtcattctgagaatagtgtatgcggcgaccgagttgctcttgcccggcgtcaatacgggataataccgcgccacatagcagaactttaaaagtgctcatcattggaaaacgttcttcggggcgaaaactctcaaggatcttaccgctgttgagatccagttcgatgtaacccactcgtgcacccaactgatcttcagcatcttttactttcaccagcgtttctgggtgagcaaaaacaggaaggcaaaatgccgcaaaaaagggaataagggcgacacggaaatgttgaatactcatactcttcctttttcaatattattgaagcatttatcagggttattgtctcatgagcggatacatatttgaatgtatttagaaaaataaacaaataggggttccgcgcacatttccccgaaaagtgccacctgacgtc